European Patent Specification EP 3 386 374 B1, published September 11, 2024. Title: Methods for Functional Brain Circuit Analysis. Applicant: Lee, Jin H. Lee, Hyun J. Weitz, Andrew J. The sequence listing filed with the application follows.

SEQUENCE LISTING (64 sequences)

SEQ ID NO: 1 - protein, 310 aa, Chlamydomonas reinhardtii
MDYGGALSAVGRELLFVTNPVVVNGSVLVPEDQCYCAGWIESRGTNGAQTASNVLQWLAAGFSILLLMFYAYQTWKSTCGWEEIYVCAIEMVKVILEFFFEFKNPSMLYLATGHRVQWLRYAEWLLTCPVILIHLSNLTGLSNDYSRRTMGLLVSDIGTIVWGATSAMATGYVKVIFFCLGLCYGANTFFHAAKAYIEGYHTVPKGRCRQVVTGMAWLFFVSWGMFPILFILGPEGFGVLSVYGSTVGHTIIDLMSKNCWGLLGHYLRVLIHEHILIHGDIRKTTKLNIGGTEIEVETLVEDEAEAGAVP

SEQ ID NO: 2 - protein, 340 aa, Artificial sequence
  Synthetic polypeptide
MDYGGALSAVGRELLFVTNPVVVNGSVLVPEDQCYCAGWIESRGTNGAQTASNVLQWLAAGFSILLLMFYAYQTWKSTCGWEEIYVCAIEMVKVILEFFFEFKNPSMLYLATGHRVQWLRYAEWLLTCPVILIHLSNLTGLSNDYSRRTMGLLVSDIGTIVWGATSAMATGYVKVIFFCLGLCYGANTFFHAAKAYIEGYHTVPKGRCRQVVTGMAWLFFVSWGMFPILFILGPEGFGVLSVYGSTVGHTIIDLMSKNCWGLLGHYLRVLIHEHILIHGDIRKTTKLNIGGTEIEVETLVEDEAEAGAVPAAAKSRITSEGEYIPLDQIDINVFCYENEV

SEQ ID NO: 3 - protein, 310 aa, Artificial sequence
  Synthetic polypeptide
MDYGGALSAVGRELLFVTNPVVVNGSVLVPEDQCYCAGWIESRGTNGAQTASNVLQWLAAGFSILLLMFYAYQTWKSTCGWEEIYVCAIEMVKVILEFFFEFKNPSMLYLATGHRVQWLRYAEWLLTSPVILIHLSNLTGLSNDYSRRTMGLLVSAIGTIVWGATSAMATGYVKVIFFCLGLCYGANTFFHAAKAYIEGYHTVPKGRCRQVVTGMAWLFFVSWGMFPILFILGPEGFGVLSVYGSTVGHTIIDLMSKNCWGLLGHYLRVLIHEHILIHGDIRKTTKLNIGGTEIEVETLVEDEAEAGAVP

SEQ ID NO: 4 - protein, 340 aa, Artificial sequence
  Synthetic polypeptide
MDYGGALSAVGRELLFVTNPVVVNGSVLVPEDQCYCAGWIESRGTNGAQTASNVLQWLAAGFSILLLMFYAYQTWKSTCGWEEIYVCAIEMVKVILEFFFEFKNPSMLYLATGHRVQWLRYAEWLLTSPVILIHLSNLTGLSNDYSRRTMGLLVSAIGTIVWGATSAMATGYVKVIFFCLGLCYGANTFFHAAKAYIEGYHTVPKGRCRQVVTGMAWLFFVSWGMFPILFILGPEGFGVLSVYGSTVGHTIIDLMSKNCWGLLGHYLRVLIHEHILIHGDIRKTTKLNIGGTEIEVETLVEDEAEAGAVPAAAKSRITSEGEYIPLDQIDINVFCYENEV

SEQ ID NO: 5 - protein, 300 aa, Volvox carteri
MDYPVARSLIVRYPTDLGNGTVCMPRGQCYCEGWLRSRGTSIEKTIAITLQWVVFALSVACLGWYAYQAWRATCGWEEVYVALIEMMKSIIEAFHEFDSPATLWLSSGNGVVWMRYGEWLLTCPVLLIHLSNLTGLKDDYSKRTMGLLVSDVGCIVWGATSAMCTGWTKILFFLISLSYGMYTYFHAAKVYIEAFHTVPKGICRELVRVMAWTFFVAWGMFPVLFLLGTEGFGHISPYGSAIGHSILDLIAKNMWGVLGNYLRVKIHEHILLYGDIRKKQKITIAGQEMEVETLVAEEED

SEQ ID NO: 6 - protein, 330 aa, Artificial sequence
  Synthetic polypeptide
MDYPVARSLIVRYPTDLGNGTVCMPRGQCYCEGWLRSRGTSIEKTIAITLQWVVFALSVACLGWYAYQAWRATCGWEEVYVALIEMMKSIIEAFHEFDSPATLWLSSGNGVVWMRYGEWLLTCPVLLIHLSNLTGLKDDYSKRTMGLLVSDVGCIVWGATSAMCTGWTKILFFLISLSYGMYTYFHAAKVYIEAFHTVPKGICRELVRVMAWTFFVAWGMFPVLFLLGTEGFGHISPYGSAIGHSILDLIAKNMWGVLGNYLRVKIHEHILLYGDIRKKQKITIAGQEMEVETLVAEEEDAAAKSRITSEGEYIPLDQIDINVFCYENEV

SEQ ID NO: 7 - protein, 344 aa, Artificial sequence
  Synthetic polypeptide
MSRRPWLLALALAVALAAGSAGASTGSDATVPVATQDGPDYVFHRAHERMLFQTSYTLENNGSVICIPNNGQCFCLAWLKSNGTNAEKLAANILQWITFALSALCLMFYGYQTWKSTCGWEEIYVATIEMIKFIIEYFHEFDEPAVIYSSNGNKTVWLRYAEWLLTCPVLLIHLSNLTGLKDDYSKRTMGLLVSDVGCIVWGATSAMCTGWTKILFFLISLSYGMYTYFHAAKVYIEAFHTVPKGICRELVRVMAWTFFVAWGMFPVLFLLGTEGFGHISPYGSAIGHSILDLIAKNMWGVLGNYLRVKIHEHILLYGDIRKKQKITIAGQEMEVETLVAEEED

SEQ ID NO: 8 - protein, 374 aa, Artificial sequence
  Synthetic polypeptide
MSRRPWLLALALAVALAAGSAGASTGSDATVPVATQDGPDYVFHRAHERMLFQTSYTLENNGSVICIPNNGQCFCLAWLKSNGTNAEKLAANILQWITFALSALCLMFYGYQTWKSTCGWEEIYVATIEMIKFIIEYFHEFDEPAVIYSSNGNKTVWLRYAEWLLTCPVLLIHLSNLTGLKDDYSKRTMGLLVSDVGCIVWGATSAMCTGWTKILFFLISLSYGMYTYFHAAKVYIEAFHTVPKGICRELVRVMAWTFFVAWGMFPVLFLLGTEGFGHISPYGSAIGHSILDLIAKNMWGVLGNYLRVKIHEHILLYGDIRKKQKITIAGQEMEVETLVAEEEDAAAKSRITSEGEYIPLDQIDINVFCYENEV

SEQ ID NO: 9 - protein, 348 aa, Artificial sequence
  Synthetic polypeptide
MSRRPWLLALALAVALAAGSAGASTGSDATVPVATQDGPDYVFHRAHERMLFQTSYTLENNGSVICIPNNGQCFCLAWLKSNGTNAEKLAANILQWITFALSALCLMFYGYQTWKSTCGWEEIYVATIEMIKFIIEYFHEFDEPAVIYSSNGNKTVWLRYAEWLLTCPVILIHLSNLTGLANDYNKRTMGLLVSDIGTIVWGTTAALSKGYVRVIFFLMGLCYGIYTFFNAAKVYIEAYHTVPKGRCRQVVTGMAWLFFVSWGMFPILFILGPEGFGVLSVYGSTVGHTIIDLMSKNCWGLLGHYLRVLIHEHILIHGDIRKTTKLNIGGTEIEVETLVEDEAEAGAV

SEQ ID NO: 10 - protein, 378 aa, Artificial sequence
  Synthetic polypeptide
MSRRPWLLALALAVALAAGSAGASTGSDATVPVATQDGPDYVFHRAHERMLFQTSYTLENNGSVICIPNNGQCFCLAWLKSNGTNAEKLAANILQWITFALSALCLMFYGYQTWKSTCGWEEIYVATIEMIKFIIEYFHEFDEPAVIYSSNGNKTVWLRYAEWLLTCPVILIHLSNLTGLANDYNKRTMGLLVSDIGTIVWGTTAALSKGYVRVIFFLMGLCYGIYTFFNAAKVYIEAYHTVPKGRCRQVVTGMAWLFFVSWGMFPILFILGPEGFGVLSVYGSTVGHTIIDLMSKNCWGLLGHYLRVLIHEHILIHGDIRKTTKLNIGGTEIEVETLVEDEAEAGAVAAAKSRITSEGEYIPLDQIDINVFCYENEV

SEQ ID NO: 11 - protein, 350 aa, Artificial sequence
  Synthetic polypeptide
MVSRRPWLLALALAVALAAGSAGASTGSDATVPVATQDGPDYVFHRAHERMLFQTSYTLENNGSVICIPNNGQCFCLAWLKSNGTNAEKLAANILQWVTFALSVACLGWYAYQAWRATCGWEEVYVALIEMMKSIIEAFHEFDSPATLWLSSGNGVVWMRYGEWLLTCPVILIHLSNLTGLKDDYSKRTMGLLVSDVGCIVWGATSAMCTGWTKILFFLISLSYGMYTYFHAAKVYIEAFHTVPKGLCRQLVRAMAWLFFVSWGMFPVLFLLGPEGFGHISPYGSAIGHSILDLIAKNMWGVLGNYLRVKIHEHILLYGDIRKKQKITIAGQEMEVETLVAEEEDKYESS

SEQ ID NO: 12 - protein, 380 aa, Artificial sequence
  Synthetic polypeptide
MVSRRPWLLALALAVALAAGSAGASTGSDATVPVATQDGPDYVFHRAHERMLFQTSYTLENNGSVICIPNNGQCFCLAWLKSNGTNAEKLAANILQWVTFALSVACLGWYAYQAWRATCGWEEVYVALIEMMKSIIEAFHEFDSPATLWLSSGNGVVWMRYGEWLLTCPVILIHLSNLTGLKDDYSKRTMGLLVSDVGCIVWGATSAMCTGWTKILFFLISLSYGMYTYFHAAKVYIEAFHTVPKGLCRQLVRAMAWLFFVSWGMFPVLFLLGPEGFGHISPYGSAIGHSILDLIAKNMWGVLGNYLRVKIHEHILLYGDIRKKQKITIAGQEMEVETLVAEEEDKYESSAAAKSRITSEGEYIPLDQIDINVFCYENEV

SEQ ID NO: 13 - protein, 316 aa, Scherffelia dubia
MGGAPAPDAHSAPPGNDSAGGSEYHAPAGYQVNPPYHPVHGYEEQCSSIYIYYGALWEQETARGFQWFAVFLSALFLAFYGWHAYKASVGWEEVYVCSVELIKVILEIYFEFTSPAMLFLYGGNITPWLRYAEWLLTCPVILIHLSNITGLSEEYNKRTMALLVSDLGTICMGVTAALATGWVKWLFYCIGLVYGTQTFYNAGIIYVESYYIMPAGGCKKLVLAMTAVYYSSWLMFPGLFIFGPEGMHTLSVAGSTIGHTIADLLSKNIWGLLGHFLRIKIHEHIIMYGDIRRPVSSQFLGRKVDVLAFVTEEDKV

SEQ ID NO: 14 - protein, 346 aa, Artificial sequence
  Synthetic polypeptide
MGGAPAPDAHSAPPGNDSAGGSEYHAPAGYQVNPPYHPVHGYEEQCSSIYIYYGALWEQETARGFQWFAVFLSALFLAFYGWHAYKASVGWEEVYVCSVELIKVILEIYFEFTSPAMLFLYGGNITPWLRYAEWLLTCPVILIHLSNITGLSEEYNKRTMALLVSDLGTICMGVTAALATGWVKWLFYCIGLVYGTQTFYNAGIIYVESYYIMPAGGCKKLVLAMTAVYYSSWLMFPGLFIFGPEGMHTLSVAGSTIGHTIADLLSKNIWGLLGHFLRIKIHEHIIMYGDIRRPVSSQFLGRKVDVLAFVTEEDKVAAAKSRITSEGEYIPLDQIDINVFCYENEV

SEQ ID NO: 15 - protein, 350 aa, Chlamydomonas noctigama
MAELISSATRSLFAAGGINPWPNPYHHEDMGCGGMTPTGECFSTEWWCDPSYGLSDAGYGYCFVEATGGYLVVGVEKKQAWLHSRGTPGEKIGAQVCQWIAFSIAIALLTFYGFSAWKATCGWEEVYVCCVEVLFVTLEIFKEFSSPATVYLSTGNHAYCLRYFEWLLSCPVILIKLSNLSGLKNDYSKRTMGLIVSCVGMIVFGMAAGLATDWLKWLLYIVSCIYGGYMYFQAAKCYVEANHSVPKGHCRMVVKLMAYAYFASWGSYPILWAVGPEGLLKLSPYANSIGHSICDIIAKEFWTFLAHHLRIKIHEHILIHGDIRKTTKMEIGGEEVEVEEFVEEEDEDTV

SEQ ID NO: 16 - protein, 380 aa, Artificial sequence
  Synthetic polypeptide
MAELISSATRSLFAAGGINPWPNPYHHEDMGCGGMTPTGECFSTEWWCDPSYGLSDAGYGYCFVEATGGYLVVGVEKKQAWLHSRGTPGEKIGAQVCQWIAFSIAIALLTFYGFSAWKATCGWEEVYVCCVEVLFVTLEIFKEFSSPATVYLSTGNHAYCLRYFEWLLSCPVILIKLSNLSGLKNDYSKRTMGLIVSCVGMIVFGMAAGLATDWLKWLLYIVSCIYGGYMYFQAAKCYVEANHSVPKGHCRMVVKLMAYAYFASWGSYPILWAVGPEGLLKLSPYANSIGHSICDIIAKEFWTFLAHHLRIKIHEHILIHGDIRKTTKMEIGGEEVEVEEFVEEEDEDTVAAAKSRITSEGEYIPLDQIDINVFCYENEV

SEQ ID NO: 17 - protein, 345 aa, Artificial sequence
  Synthetic polypeptide
MSRLVAASWLLALLLCGITSTTTASSAPAASSTDGTAAAAVSHYAMNGFDELAKGAVVPEDHFVCGPADKCYCSAWLHSRGTPGEKIGAQVCQWIAFSIAIALLTFYGFSAWKATCGWEEVYVCCVEVLFVTLEIFKEFSSPATVYLSTGNHAYCLRYFEWLLSCPVILIKLSNLSGLKNDYSKRTMGLIVSCVGMIVFGMAAGLATDWLKWLLYIVSCIYGGYMYFQAAKCYVEANHSVPKGHCRMVVKLMAYAYFASWGSYPILWAVGPEGLLKLSPYANSIGHSICDIIAKEFWTFLAHHLRIKIHEHILIHGDIRKTTKMEIGGEEVEVEEFVEEEDEDTV

SEQ ID NO: 18 - protein, 375 aa, Artificial sequence
  Synthetic polypeptide
MSRLVAASWLLALLLCGITSTTTASSAPAASSTDGTAAAAVSHYAMNGFDELAKGAVVPEDHFVCGPADKCYCSAWLHSRGTPGEKIGAQVCQWIAFSIAIALLTFYGFSAWKATCGWEEVYVCCVEVLFVTLEIFKEFSSPATVYLSTGNHAYCLRYFEWLLSCPVILIKLSNLSGLKNDYSKRTMGLIVSCVGMIVFGMAAGLATDWLKWLLYIVSCIYGGYMYFQAAKCYVEANHSVPKGHCRMVVKLMAYAYFASWGSYPILWAVGPEGLLKLSPYANSIGHSICDIIAKEFWTFLAHHLRIKIHEHILIHGDIRKTTKMEIGGEEVEVEEFVEEEDEDTVAAAKSRITSEGEYIPLDQIDINVFCYENEV

SEQ ID NO: 19 - protein, 325 aa, Stigeoclonium helveticum
METAATMTHAFISAVPSAEATIRGLLSAAAVVTPAADAHGETSNATTAGADHGCFPHINHGTELQHKIAVGLQWFTVIVAIVQLIFYGWHSFKATTGWEEVYVCVIELVKCFIELFHEVDSPATVYQTNGGAVIWLRYSMWLLTCPVILIHLSNLTGLHEEYSKRTMTILVTDIGNIVWGITAAFTKGPLKILFFMIGLFYGVTCFFQIAKVYIESYHTLPKGVCRKICKIMAYVFFCSWLMFPVMFIAGHEGLGLITPYTSGIGHLILDLISKNTWGFLGHHLRVKIHEHILIHGDIRKTTTINVAGENMEIETFVDEEEEGGV

SEQ ID NO: 20 - protein, 355 aa, Artificial sequence
  Synthetic polypeptide
METAATMTHAFISAVPSAEATIRGLLSAAAVVTPAADAHGETSNATTAGADHGCFPHINHGTELQHKIAVGLQWFTVIVAIVQLIFYGWHSFKATTGWEEVYVCVIELVKCFIELFHEVDSPATVYQTNGGAVIWLRYSMWLLTCPVILIHLSNLTGLHEEYSKRTMTILVTDIGNIVWGITAAFTKGPLKILFFMIGLFYGVTCFFQIAKVYIESYHTLPKGVCRKICKIMAYVFFCSWLMFPVMFIAGHEGLGLITPYTSGIGHLILDLISKNTWGFLGHHLRVKIHEHILIHGDIRKTTTINVAGENMEIETFVDEEEEGGVAAAKSRITSEGEYIPLDQIDINVFCYENEV

SEQ ID NO: 21 - protein, 258 aa, Halorubrum sodomense
MDPIALQAGYDLLGDGRPETLWLGIGTLLMLIGTFYFLVRGWGVTDKDAREYYAVTILVPGIASAAYLSMFFGIGLTEVTVGGEMLDIYYARYADWLFTTPLLLLDLALLAKVDRVTIGTLVGVDALMIVTGLIGALSHTAIARYSWWLFSTICMIVVLYFLATSLRSAAKERGPEVASTFNTLTALVLVLWTAYPILWIIGTEGAGVVGLGIETLLFMVLDVTAKVGFGFILLRSRAILGDTEAPEPSAGADVSAAD

SEQ ID NO: 22 - protein, 293 aa, Artificial sequence
  Synthetic polypeptide
MDPIALQAGYDLLGDGRPETLWLGIGTLLMLIGTFYFLVRGWGVTDKDAREYYAVTILVPGIASAAYLSMFFGIGLTEVTVGGEMLDIYYARYADWLFTTPLLLLDLALLAKVDRVTIGTLVGVDALMIVTGLIGALSHTAIARYSWWLFSTICMIVVLYFLATSLRSAAKERGPEVASTFNTLTALVLVLWTAYPILWIIGTEGAGVVGLGIETLLFMVLDVTAKVGFGFILLRSRAILGDTEAPEPSAGADVSAADRPVVAAAAKSRITSEGEYIPLDQIDINVFCYENEV

SEQ ID NO: 23 - protein, 248 aa, Halorubrum sp. TP009
MDPIALQAGYDLLGDGRPETLWLGIGTLLMLIGTFYFIVKGWGVTDKEAREYYSITILVPGIASAAYLSMFFGIGLTEVTVAGEVLDIYYARYADWLFTTPLLLLDLALLAKVDRVSIGTLVGVDALMIVTGLIGALSHTPLARYSWWLFSTICMIVVLYFLATSLRAAAKERGPEVASTFNTLTALVLVLWTAYPILWIIGTEGAGVVGLGIETLLFMVLDVTAKVGFGFILLRSRAILGDTEAPEP

SEQ ID NO: 24 - protein, 278 aa, Artificial sequence
  Synthetic polypeptide
MDPIALQAGYDLLGDGRPETLWLGIGTLLMLIGTFYFIVKGWGVTDKEAREYYSITILVPGIASAAYLSMFFGIGLTEVTVAGEVLDIYYARYADWLFTTPLLLLDLALLAKVDRVSIGTLVGVDALMIVTGLIGALSHTPLARYSWWLFSTICMIVVLYFLATSLRAAAKERGPEVASTFNTLTALVLVLWTAYPILWIIGTEGAGVVGLGIETLLFMVLDVTAKVGFGFILLRSRAILGDTEAPEPAAAKSRITSEGEYIPLDQIDINVFCYENEV

SEQ ID NO: 25 - protein, 242 aa, Guillardia theta
MLVGEGAKLDVHGCKTVDMASSFGKALLEFVFIVFACITLLLGINAAKSKAASRVLFPATFVTGIASIAYFSMASGGGWVIAPDCRQLFVARYLDWLITTPLLLIDLGLVAGVSRWDIMALCLSDVLMIATGAFGSLTVGNVKWVWWFFGMCWFLHIIFALGKSWAEAAKAKGGDSASVYSKIAGITVITWFCYPVVWVFAEGFGNFSVTFEVLIYGVLDVISKAVFGLILMSGAATGYESI

SEQ ID NO: 26 - protein, 272 aa, Artificial sequence
  Synthetic polypeptide
MLVGEGAKLDVHGCKTVDMASSFGKALLEFVFIVFACITLLLGINAAKSKAASRVLFPATFVTGIASIAYFSMASGGGWVIAPDCRQLFVARYLDWLITTPLLLIDLGLVAGVSRWDIMALCLSDVLMIATGAFGSLTVGNVKWVWWFFGMCWFLHIIFALGKSWAEAAKAKGGDSASVYSKIAGITVITWFCYPVVWVFAEGFGNFSVTFEVLIYGVLDVISKAVFGLILMSGAATGYESIAAAKSRITSEGEYIPLDQIDINVFCYENEV

SEQ ID NO: 27 - protein, 262 aa, Oxyrrhis marina
MAPLAQDWTYAEWSAVYNALSFGIAGMGSATIFFWLQLPNVTKNYRTALTITGIVTLIATYHYFRIFNSWVAAFNVGLGVNGAYEVTVSGTPFNDAYRYVDWLLTVPLLLVELILVMKLPAKETVCLAWTLGIASAVMVALGYPGEIQDDLSVRWFWWACAMVPFVYVVGTLVVGLGAATAKQPEGVVDLVSAARYLTVVSWLTYPFVYIVKNIGLAGSTATMYEQIGYSAADVTAKAVFGVLIWAIANAKSRLEEEGKLRA

SEQ ID NO: 28 - protein, 292 aa, Artificial sequence
  Synthetic polypeptide
MAPLAQDWTYAEWSAVYNALSFGIAGMGSATIFFWLQLPNVTKNYRTALTITGIVTLIATYHYFRIFNSWVAAFNVGLGVNGAYEVTVSGTPFNDAYRYVDWLLTVPLLLVELILVMKLPAKETVCLAWTLGIASAVMVALGYPGEIQDDLSVRWFWWACAMVPFVYVVGTLVVGLGAATAKQPEGVVDLVSAARYLTVVSWLTYPFVYIVKNIGLAGSTATMYEQIGYSAADVTAKAVFGVLIWAIANAKSRLEEEGKLRAAAAKSRITSEGEYIPLDQIDINVFCYENEV

SEQ ID NO: 29 - protein, 313 aa, Leptosphaeria maculans
MIVDQFEEVLMKTSQLFPLPTATQSAQPTHVAPVPTVLPDTPIYETVGDSGSKTLWVVFVLMLIASAAFTALSWKIPVNRRLYHVITTIITLTAALSYFAMATGHGVALNKIVIRTQHDHVPDTYETVYRQVYYARYIDWAITTPLLLLDLGLLAGMSGAHIFMAIVADLIMVLTGLFAAFGSEGTPQKWGWYTIACIAYIFVVWHLVLNGGANARVKGEKLRSFFVAIGAYTLILWTAYPIVWGLADGARKIGVDGEIIAYAVLDVLAKGVFGAWLLVTHANLRESDVELNGFWANGLNREGAIRIGEDDGA

SEQ ID NO: 30 - protein, 351 aa, Artificial sequence
  Synthetic polypeptide
MIVDQFEEVLMKTSQLFPLPTATQSAQPTHVAPVPTVLPDTPIYETVGDSGSKTLWVVFVLMLIASAAFTALSWKIPVNRRLYHVITTIITLTAALSYFAMATGHGVALNKIVIRTQHDHVPDTYETVYRQVYYARYIDWAITTPLLLLDLGLLAGMSGAHIFMAIVADLIMVLTGLFAAFGSEGTPQKWGWYTIACIAYIFVVWHLVLNGGANARVKGEKLRSFFVAIGAYTLILWTAYPIVWGLADGARKIGVDGEIIAYAVLDVLAKGVFGAWLLVTHANLRESDVELNGFWANGLNREGAIRIGEDDGARPVVAVSKAAAKSRITSEGEYIPLDQIDINVFCYENEV

SEQ ID NO: 31 - protein, 291 aa, Natronomonas pharaonis
MTETLPPVTESAVALQAEVTQRELFEFVLNDPLLASSLYINIALAGLSILLFVFMTRGLDDPRAKLIAVSTILVPVVSIASYTGLASGLTISVLEMPAGHFAEGSSVMLGGEEVDGVVTMWGRYLTWALSTPMILLALGLLAGSNATKLFTAITFDIAMCVTGLAAALTTSSHLMRWFWYAISCACFLVVLYILLVEWAQDAKAAGTADMFNTLKLLTVVMWLGYPIVWALGVEGIAVLPVGVTSWGYSFLDIVAKYIFAFLLLNYLTSNESVVSGSILDVPSASGTPADD

SEQ ID NO: 32 - protein, 320 aa, Artificial sequence
  Synthetic polypeptide
MTETLPPVTESAVALQAEVTQRELFEFVLNDPLLASSLYINIALAGLSILLFVFMTRGLDDPRAKLIAVSTILVPVVSIASYTGLASGLTISVLEMPAGHFAEGSSVMLGGEEVDGVVTMWGRYLTWALSTPMILLALGLLAGSNATKLFTAITFDIAMCVTGLAAALTTSSHLMRWFWYAISCACFLVVLYILLVEWAQDAKAAGTADMFNTLKLLTVVMWLGYPIVWALGVEGIAVLPVGVTSWGYSFLDIVAKYIFAFLLLNYLTSNESVVSGSILDVPSASGTPADDAAAKSRITSEGEYIPLDQIDINFCYENEV

SEQ ID NO: 33 - protein, 303 aa, Artificial sequence
  Synthetic polypeptide
MVTQRELFEFVLNDPLLASSLYINIALAGLSILLFVFMTRGLDDPRAKLIAVSTILVPVVSIASYTGLASGLTISVLEMPAGHFAEGSSVMLGGEEVDGVVTMWGRYLTWALSTPMILLALGLLAGSNATKLFTAITFDIAMCVTGLAAALTTSSHLMRWFWYAISCACFLVVLYILLVEWAQDAKAAGTADMFNTLKLLTVVMWLGYPIVWALGVEGIAVLPVGVTSWGYSFLDIVAKYIFAFLLLNYLTSNESVVSGSILDVPSASGTPADDAAAKSRITSEGEYIPLDQIDINFCYENEV

SEQ ID NO: 34 - protein, 365 aa, Dunaliella salina
MRRRESQLAYLCLFVLIAGWAPRLTESAPDLAERRPPSERNTPYANIKKVPNITEPNANVQLDGWALYQDFYYLAGSDKEWVVGPSDQCYCRAWSKSHGTDREGEAAVVWAYIVFAICIVQLVYFMFAAWKATVGWEEVYVNIIELVHIALVIWVEFDKPAMLYLNDGQMVPWLRYSAWLLSCPVILIHLSNLTGLKGDYSKRTMGLLVSDIGTIVFGTSAALAPPNHVKVILFTIGLLYGLFTFFTAAKVYIEAYHTVPKGQCRNLVRAMAWTYFVSWAMFPILFILGREGFGHITYFGSSIGHFILEIFSKNLWSLLGHGLRYRIRQHIIIHGNLTKKNKINIAGDNVEVEEYVDSNDKDSDV

SEQ ID NO: 35 - protein, 395 aa, Artificial sequence
  Synthetic polypeptide
MRRRESQLAYLCLFVLIAGWAPRLTESAPDLAERRPPSERNTPYANIKKVPNITEPNANVQLDGWALYQDFYYLAGSDKEWVVGPSDQCYCRAWSKSHGTDREGEAAVVWAYIVFAICIVQLVYFMFAAWKATVGWEEVYVNIIELVHIALVIWVEFDKPAMLYLNDGQMVPWLRYSAWLLSCPVILIHLSNLTGLKGDYSKRTMGLLVSDIGTIVFGTSAALAPPNHVKVILFTIGLLYGLFTFFTAAKVYIEAYHTVPKGQCRNLVRAMAWTYFVSWAMFPILFILGREGFGHITYFGSSIGHFILEIFSKNLWSLLGHGLRYRIRQHIIIHGNLTKKNKINIAGDNVEVEEYVDSNDKDSDVAAAKSRITSEGEYIPLDQIDINVFCYENEV

SEQ ID NO: 36 - protein, 348 aa, Artificial sequence
  Synthetic polypeptide
MSRRPWLLALALAVALAAGSAGASTGSDATVPVATQDGPDYVFHRAHERMLFQTSYTLENNGSVICIPNNGQCFCLAWLKSNGTNAEKLAANILQWISFALSALCLMFYGYQTWKSTCGWEEIYVATISMIKFIIEYFHSFDEPAVIYSSNGNKTKWLRYASWLLTCPVILIRLSNLTGLANDYNKRTMGLLVSDIGTIVWGTTAALSKGYVRVIFFLMGLCYGIYTFFNAAKVYIEAYHTVPKGRCRQVVTGMAWLFFVSWGMFPILFILGPEGFGVLSKYGSNVGHTIIDLMSKQCWGLLGHYLRVLIHEHILIHGDIRKTTKLNIGGTEIEVETLVEDEAEAGAV

SEQ ID NO: 37 - protein, 378 aa, Artificial sequence
  Synthetic polypeptide
MSRRPWLLALALAVALAAGSAGASTGSDATVPVATQDGPDYVFHRAHERMLFQTSYTLENNGSVICIPNNGQCFCLAWLKSNGTNAEKLAANILQWISFALSALCLMFYGYQTWKSTCGWEEIYVATISMIKFIIEYFHSFDEPAVIYSSNGNKTKWLRYASWLLTCPVILIRLSNLTGLANDYNKRTMGLLVSDIGTIVWGTTAALSKGYVRVIFFLMGLCYGIYTFFNAAKVYIEAYHTVPKGRCRQVVTGMAWLFFVSWGMFPILFILGPEGFGVLSKYGSNVGHTIIDLMSKQCWGLLGHYLRVLIHEHILIHGDIRKTTKLNIGGTEIEVETLVEDEAEAGAVAAAKSRITSEGEYIPLDQIDINVFCYENEV

SEQ ID NO: 38 - protein, 348 aa, Artificial sequence
  Synthetic polypeptide
  MISC_FEATURE (167)..(167): Xaa may be Thr or Ser.
MSRRPWLLALALAVALAAGSAGASTGSDATVPVATQDGPDYVFHRAHERMLFQTSYTLENNGSVICIPNNGQCFCLAWLKSNGTNAEKLAANILQWISFALSALCLMFYGYQTWKSTCGWEEIYVATISMIKFIIEYFHSFDEPAVIYSSNGNKTKWLRYASWLLTXPVILIRLSNLTGLANDYNKRTMGLLVSDIGTIVWGTTAALSKGYVRVIFFLMGLCYGIYTFFNAAKVYIEAYHTVPKGRCRQVVTGMAWLFFVSWGMFPILFILGPEGFGVLSKYGSNVGHTIIDLMSKQCWGLLGHYLRVLIHEHILIHGDIRKTTKLNIGGTEIEVETLVEDEAEAGAV

SEQ ID NO: 39 - protein, 378 aa, Artificial sequence
  Synthetic polypeptide
  MISC_FEATURE (167)..(167): Xaa may be Thr or Ser.
MSRRPWLLALALAVALAAGSAGASTGSDATVPVATQDGPDYVFHRAHERMLFQTSYTLENNGSVICIPNNGQCFCLAWLKSNGTNAEKLAANILQWISFALSALCLMFYGYQTWKSTCGWEEIYVATISMIKFIIEYFHSFDEPAVIYSSNGNKTKWLRYASWLLTXPVILIRLSNLTGLANDYNKRTMGLLVSDIGTIVWGTTAALSKGYVRVIFFLMGLCYGIYTFFNAAKVYIEAYHTVPKGRCRQVVTGMAWLFFVSWGMFPILFILGPEGFGVLSKYGSNVGHTIIDLMSKQCWGLLGHYLRVLIHEHILIHGDIRKTTKLNIGGTEIEVETLVEDEAEAGAVAAAKSRITSEGEYIPLDQIDINVFCYENEV

SEQ ID NO: 40 - protein, 309 aa, Artificial sequence
  Synthetic polypeptide
MDYGGALSAVGLFQTSYTLENNGSVICIPNNGQCFCLAWLKSNGTNAEKLAANILQWISFALSALCLMFYGYQTWKSTCGWEEIYVATISMIKFIIEYFHSFDEPAVIYSSNGNKTKWLRYASWLLTCPVILIRLSNLTGLANDYNKRTMGLLVSDIGTIVWGTTAALSKGYVRVIFFLMGLCYGIYTFFNAAKVYIEAYHTVPKGRCRQVVTGMAWLFFVSWGMFPILFILGPEGFGVLSKYGSNVGHTIIDLMSKQCWGLLGHYLRVLIHEHILIHGDIRKTTKLNIGGTEIEVETLVEDEAEAGAV

SEQ ID NO: 41 - protein, 339 aa, Artificial sequence
  Synthetic polypeptide
MDYGGALSAVGLFQTSYTLENNGSVICIPNNGQCFCLAWLKSNGTNAEKLAANILQWISFALSALCLMFYGYQTWKSTCGWEEIYVATISMIKFIIEYFHSFDEPAVIYSSNGNKTKWLRYASWLLTCPVILIRLSNLTGLANDYNKRTMGLLVSDIGTIVWGTTAALSKGYVRVIFFLMGLCYGIYTFFNAAKVYIEAYHTVPKGRCRQVVTGMAWLFFVSWGMFPILFILGPEGFGVLSKYGSNVGHTIIDLMSKQCWGLLGHYLRVLIHEHILIHGDIRKTTKLNIGGTEIEVETLVEDEAEAGAVAAAKSRITSEGEYIPLDQIDINVFCYENEV

SEQ ID NO: 42 - protein, 310 aa, Artificial sequence
  Synthetic polypeptide
MDYGGALSAVGRELLFVTNPVVVNGSVLVPEDQCYCAGWIESRGTNGAQTASNVLQWLSAGFSILLLMFYAYQTWKSTCGWEEIYVCAISMVKVILEFFFSFKNPSMLYLATGHRVKWLRYASWLLTCPVILIRLSNLTGLSNDYSRRTMGLLVSDIGTIVWGATSAMATGYVKVIFFCLGLCYGANTFFHAAKAYIEGYHTVPKGRCRQVVTGMAWLFFVSWGMFPILFILGPEGFGVLSKYGSNVGHTIIDLMSKQCWGLLGHYLRVLIHEHILIHGDIRKTTKLNIGGTEIEVETLVEDEAEAGAVP

SEQ ID NO: 43 - protein, 340 aa, Artificial sequence
  Synthetic polypeptide
MDYGGALSAVGRELLFVTNPVVVNGSVLVPEDQCYCAGWIESRGTNGAQTASNVLQWLSAGFSILLLMFYAYQTWKSTCGWEEIYVCAISMVKVILEFFFSFKNPSMLYLATGHRVKWLRYASWLLTCPVILIRLSNLTGLSNDYSRRTMGLLVSDIGTIVWGATSAMATGYVKVIFFCLGLCYGANTFFHAAKAYIEGYHTVPKGRCRQVVTGMAWLFFVSWGMFPILFILGPEGFGVLSKYGSNVGHTIIDLMSKQCWGLLGHYLRVLIHEHILIHGDIRKTTKLNIGGTEIEVETLVEDEAEAGAVPAAAKSRITSEGEYIPLDQIDINVFCYENEV

SEQ ID NO: 44 - protein, 344 aa, Artificial sequence
  Synthetic polypeptide
MSRRPWLLALALAVALAAGSAGASTGSDATVPVATQDGPDYVFHRAHERMLFQTSYTLENNGSVICIPNNGQCFCLAWLKSNGTNAEKLAANILQWISFALSALCLMFYGYQTWKSTCGWEEIYVATISMIKFIIEYFHSFDEPAVIYSSNGNKTKWLRYASWLLTCPVLLIRLSNLTGLKDDYSKRTMGLLVSDVGCIVWGATSAMCTGWTKILFFLISLSYGMYTYFHAAKVYIEAFHTVPKGICRELVRVMAWTFFVAWGMFPVLFLLGTEGFGHISKYGSNIGHSILDLIAKQMWGVLGNYLRVKIHEHILLYGDIRKKQKITIAGQEMEVETLVAEEED

SEQ ID NO: 45 - protein, 374 aa, Artificial sequence
  Synthetic polypeptide
MSRRPWLLALALAVALAAGSAGASTGSDATVPVATQDGPDYVFHRAHERMLFQTSYTLENNGSVICIPNNGQCFCLAWLKSNGTNAEKLAANILQWISFALSALCLMFYGYQTWKSTCGWEEIYVATISMIKFIIEYFHSFDEPAVIYSSNGNKTKWLRYASWLLTCPVLLIRLSNLTGLKDDYSKRTMGLLVSDVGCIVWGATSAMCTGWTKILFFLISLSYGMYTYFHAAKVYIEAFHTVPKGICRELVRVMAWTFFVAWGMFPVLFLLGTEGFGHISKYGSNIGHSILDLIAKQMWGVLGNYLRVKIHEHILLYGDIRKKQKITIAGQEMEVETLVAEEEDAAAKSRITSEGEYIPLDQIDINVFCYENEV

SEQ ID NO: 46 - protein, 305 aa, Artificial sequence
  Synthetic polypeptide
MDYGGALSAVGLFQTSYTLENNGSVICIPNNGQCFCLAWLKSNGTNAEKLAANILQWISFALSALCLMFYGYQTWKSTCGWEEIYVATISMIKFIIEYFHSFDEPAVIYSSNGNKTKWLRYASWLLTCPVLLIRLSNLTGLKDDYSKRTMGLLVSDVGCIVWGATSAMCTGWTKILFFLISLSYGMYTYFHAAKVYIEAFHTVPKGICRELVRVMAWTFFVAWGMFPVLFLLGTEGFGHISKYGSNIGHSILDLIAKQMWGVLGNYLRVKIHEHILLYGDIRKKQKITIAGQEMEVETLVAEEED

SEQ ID NO: 47 - protein, 335 aa, Artificial sequence
  Synthetic polypeptide
MDYGGALSAVGLFQTSYTLENNGSVICIPNNGQCFCLAWLKSNGTNAEKLAANILQWISFALSALCLMFYGYQTWKSTCGWEEIYVATISMIKFIIEYFHSFDEPAVIYSSNGNKTKWLRYASWLLTCPVLLIRLSNLTGLKDDYSKRTMGLLVSDVGCIVWGATSAMCTGWTKILFFLISLSYGMYTYFHAAKVYIEAFHTVPKGICRELVRVMAWTFFVAWGMFPVLFLLGTEGFGHISKYGSNIGHSILDLIAKQMWGVLGNYLRVKIHEHILLYGDIRKKQKITIAGQEMEVETLVAEEEDAAAKSRITSEGEYIPLDQIDINVFCYENEV

SEQ ID NO: 48 - protein, 350 aa, Artificial sequence
  Synthetic polypeptide
MVSRRPWLLALALAVALAAGSAGASTGSDATVPVATQDGPDYVFHRAHERMLFQTSYTLENNGSVICIPNNGQCFCLAWLKSNGTNAEKLAANILQWVSFALSVACLGWYAYQAWRATCGWEEVYVALISMMKSIIEAFHSFDSPATLWLSSGNGVKWMRYGSWLLTCPVILIRLSNLTGLKDDYSKRTMGLLVSDVGCIVWGATSAMCTGWTKILFFLISLSYGMYTYFHAAKVYIEAFHTVPKGLCRQLVRAMAWLFFVSWGMFPVLFLLGPEGFGHISKYGSNIGHSILDLIAKQMWGVLGNYLRVKIHEHILLYGDIRKKQKITIAGQEMEVETLVAEEEDKYESS

SEQ ID NO: 49 - protein, 380 aa, Artificial sequence
  Synthetic polypeptide
MVSRRPWLLALALAVALAAGSAGASTGSDATVPVATQDGPDYVFHRAHERMLFQTSYTLENNGSVICIPNNGQCFCLAWLKSNGTNAEKLAANILQWVSFALSVACLGWYAYQAWRATCGWEEVYVALISMMKSIIEAFHSFDSPATLWLSSGNGVKWMRYGSWLLTCPVILIRLSNLTGLKDDYSKRTMGLLVSDVGCIVWGATSAMCTGWTKILFFLISLSYGMYTYFHAAKVYIEAFHTVPKGLCRQLVRAMAWLFFVSWGMFPVLFLLGPEGFGHISKYGSNIGHSILDLIAKQMWGVLGNYLRVKIHEHILLYGDIRKKQKITIAGQEMEVETLVAEEEDKYESSAAAKSRITSEGEYIPLDQIDINVFCYENEV

SEQ ID NO: 50 - protein, 310 aa, Artificial sequence
  Synthetic polypeptide
MDYGGALSAVGLFQTSYTLENNGSVICIPNNGQCFCLAWLKSNGTNAEKLAANILQWVSFALSVACLGWYAYQAWRATCGWEEVYVALISMMKSIIEAFHSFDSPATLWLSSGNGVKWMRYGSWLLTCPVILIRLSNLTGLKDDYSKRTMGLLVSDVGCIVWGATSAMCTGWTKILFFLISLSYGMYTYFHAAKVYIEAFHTVPKGLCRQLVRAMAWLFFVSWGMFPVLFLLGPEGFGHISKYGSNIGHSILDLIAKQMWGVLGNYLRVKIHEHILLYGDIRKKQKITIAGQEMEVETLVAEEEDKYESS

SEQ ID NO: 51 - protein, 340 aa, Artificial sequence
  Synthetic polypeptide
MDYGGALSAVGLFQTSYTLENNGSVICIPNNGQCFCLAWLKSNGTNAEKLAANILQWVSFALSVACLGWYAYQAWRATCGWEEVYVALISMMKSIIEAFHSFDSPATLWLSSGNGVKWMRYGSWLLTCPVILIRLSNLTGLKDDYSKRTMGLLVSDVGCIVWGATSAMCTGWTKILFFLISLSYGMYTYFHAAKVYIEAFHTVPKGLCRQLVRAMAWLFFVSWGMFPVLFLLGPEGFGHISKYGSNIGHSILDLIAKQMWGVLGNYLRVKIHEHILLYGDIRKKQKITIAGQEMEVETLVAEEEDKYESSAAAKSRITSEGEYIPLDQIDINVFCYENEV

SEQ ID NO: 52 - protein, 5 aa, Artificial sequence
  Synthetic polypeptide
  MISC_FEATURE (2)..(2): Xaa may be any amino acid.
  MISC_FEATURE (3)..(3): Xaa may be any amino acid.
VXXSL

SEQ ID NO: 53 - protein, 5 aa, Artificial sequence
  Synthetic polypeptide
VKESL

SEQ ID NO: 54 - protein, 5 aa, Artificial sequence
  Synthetic polypeptide
VLGSL

SEQ ID NO: 55 - protein, 16 aa, Artificial sequence
  Synthetic polypeptide
NANSFCYENEVALTSK

SEQ ID NO: 56 - protein, 20 aa, Artificial sequence
  Synthetic polypeptide
KSRITSEGEYIPLDQIDINV

SEQ ID NO: 57 - protein, 6 aa, Artificial sequence
  Synthetic polypeptide
  MISC_FEATURE (2)..(2): Xaa may be any amino acid.
FXYENE

SEQ ID NO: 58 - protein, 7 aa, Artificial sequence
  Synthetic polypeptide
FCYENEV

SEQ ID NO: 59 - protein, 26 aa, Artificial sequence
  Synthetic polypeptide
MDYGGALSAVGRELLFVTNPVVVNGS

SEQ ID NO: 60 - protein, 27 aa, Artificial sequence
  Synthetic polypeptide
MAGHSNSMALFSFSLLWLCSGVLGTEF

SEQ ID NO: 61 - protein, 18 aa, Artificial sequence
  Synthetic polypeptide
MRGTPLLLVVSLFSLLQD

SEQ ID NO: 62 - protein, 18 aa, Artificial sequence
  Synthetic polypeptide
MTETLPPVTESAVALQAE

SEQ ID NO: 63 - protein, 11 aa, Artificial sequence
  Synthetic polypeptide
MDYGGALSAVG

SEQ ID NO: 64 - protein, 23 aa, Artificial sequence
  Synthetic polypeptide
MGLRALMLWLLAAAGLVRESLQG